European Patent Application EP 4 129 346 A1, published February 8, 2023. Title: Mutant Viral Capsid Libraries and Related Systems and Methods. Applicant: Adverum Biotechnologies, Inc. The sequence listing filed with the application follows.

SEQUENCE LISTING (6 sequences)

SEQ ID NO: 1 - DNA, 91 bp, Streptomyces phage phiC31
gtcagaagcggttttcgggagtagtgccccaactggggtaacctttgagttctctcagttgggggcgtagggtcgccgacatgacacaagg

SEQ ID NO: 2 - DNA, 90 bp, Streptomyces sp.
gacggtctcgaagccgcggtgcgggtgccagggcgtgcccttgggctccccgggcgcgtactccacctcacccatctggtccatcatgat

SEQ ID NO: 3 - DNA, 90 bp, Mycobacterium phage Bxb1
cgtgatgacctgtgtcttcgtggtttgtctggtcaaccaccgcggtctcagtggtgtacggtacaaacccatgagagccctggtagtcat

SEQ ID NO: 4 - DNA, 40 bp, Mycobacterium sp.
ccggcttgtcgacgacggcggtctccgtcgtcaggatcat

SEQ ID NO: 5 - DNA, 90 bp, Lactococcus phage TP901-1
agatatcatatttaaattccaactcgcttaattgcgagtttttatttcgtttatttcaattaaggtaactaaaaaactccttttaaggag

SEQ ID NO: 6 - DNA, 90 bp, Lactococcus sp.
ttaaaatactgataattgccaacacaattaacatctcaatcaaggtaaatgctttttgctttttttgccaaagctttcttccgtgaattt